European Patent Application EP 4 324 925 A1, published February 21, 2024. Title: ANTI-C1S ANTIBODY. Applicant: CHUGAI SEIYAKU KABUSHIKI KAISHA. The sequence listing filed with the application follows.

SEQUENCE LISTING (89 sequences)

SEQ ID NO: 1 - protein, 673 aa, Homo sapiens
EPTMYGEILSPNYPQAYPSEVEKSWDIEVPEGYGIHLYFTHLDIELSENCAYDSVQIISGDTEEGRLCGQRSSNNPHSPIVEEFQVPYNKLQVIFKSDFSNEERFTGFAAYYVATDINECTDFVDVPCSHFCNNFIGGYFCSCPPEYFLHDDMKNCGVNCSGDVFTALIGEIASPNYPKPYPENSRCEYQIRLEKGFQVVVTLRREDFDVEAADSAGNCLDSLVFVAGDRQFGPYCGHGFPGPLNIETKSNALDIIFQTDLTGQKKGWKLRYHGDPMPCPKEDTPNSVWEPAKAKYVFRDVVQITCLDGFEVVEGRVGATSFYSTCQSNGKWSNSKLKCQPVDCGIPESIENGKVEDPESTLFGSVIRYTCEEPYYYMENGGGGEYHCAGNGSWVNEVLGPELPKCVPVCGVPREPFEEKQRIIGGSDADIKNFPWQVFFDNPWAGGALINEYWVLTAAHVVEGNREPTMYVGSTSVQTSRLAKSKMLTPEHVFIHPGWKLLEVPEGRTNFDNDIALVRLKDPVKMGPTVSPICLPGTSSDYNLMDGDLGLISGWGRTEKRDRAVRLKAARLPVAPLRKCKEVKVEKPTADAEAYVFTPNMICAGGEKGMDSCKGDSGGAFAVQDPNDKTKFYAAGLVSWGPQCGTYGLYTRVKNYVDWIMKTMQENSTPRED

SEQ ID NO: 2 - protein, 688 aa, Homo sapiens
SIPIPQKLFGEVTSPLFPKPYPNNFETTTVITVPTGYRVKLVFQQFDLEPSEGCFYDYVKISADKKSLGRFCGQLGSPLGNPPGKKEFMSQGNKMLLTFHTDFSNEENGTIMFYKGFLAYYQAVDLDECASRSKLGEEDPQPQCQHLCHNYVGGYFCSCRPGYELQEDRHSCQAECSSELYTEASGYISSLEYPRSYPPDLRCNYSIRVERGLTLHLKFLEPFDIDDHQQVHCPYDQLQIYANGKNIGEFCGKQRPPDLDTSSNAVDLLFFTDESGDSRGWKLRYTTEIIKCPQPKTLDEFTIIQNLQPQYQFRDYFIATCKQGYQLIEGNQVLHSFTAVCQDDGTWHRAMPRCKIKDCGQPRNLPNGDFRYTTTMGVNTYKARIQYYCHEPYYKMQTRAGSRESEQGVYTCTAQGIWKNEQKGEKIPRCLPVCGKPVNPVEQRQQIIGGQKAKMGNFPWQVFTNIHGRGGGALLGDRWILTAAHTLYPKEHEAQSNASLDVFLGHTNVEELMKLGNHPIRRVSVHPDYRQDESYNFEGDIALLELENSVTLGPNLLPICLPDNDTFYDLGLMGYVSGFGVMEEKIAHDLRFVRLPVANPQACENWLRGKNRMDVFSQNMFCAGHPSLKQDACQGDAGGVFAVRDPNTDRWVATGIVSWGIGCSRGYGFYTKVLNYVDWIKKEMEEED

SEQ ID NO: 3 - protein, 673 aa, Macaca fascicularis
EPTMYGEILSPNYPQAYPSEVEKSWDIEVPEGYGIHLYFTHLDIELSENCAYDSVQIMSGDIEEGRLCGQRTSNNPHSPIVEEFQVPYNKLQVIFKSDFSNEERFTGFAAYYVATDINECTDFVDAPCSHFCNNFIGGYFCSCPPEYFLHDDMKNCGVNCSGDVFTALIGEIASPNYPKPYPENSRCEYQIRLEKGFQVVVTVRREDFDVEPADSEGNCLDSLVFVAGDQQFGPYCGRGFPGPLNIETKSNALDIIFQTDLTGQNKGWKLRYHGDPMPCPKEETPTSVWEPAKAKYVFRDVVRITCLDGFEVVEGRVGATSFHSTCQSNGKWSNSKLKCQPVDCGIPESIENGKVEDPESTLFGSVTRYTCEEPYYYMENGGNGQYHCASNGSWVNEALSPELPKCVPVCGVPREPFEGKQRIIGGSDADIKNFPWQVFFDNPWAGGALIDEYWVLTAAHVVEGNQEPTMYVGSTSVQTSRLAKSKMLTSERVFIHPGWKLLEVPEARTNFDNDIALVQLKDPVKMGPTVAPICLPGTSSDYNLMDGDLGLIAGWGRTEKRDRALRLKAARLPVAPLRKCREVKVENPKADAGAYVFTPNMICAGGEKGMDSCKGDSGGAFAVQDPNDKAKFYVAGLVSWGPQCGTYGLYTRVQNYVDWIKKTMQENSTPSKD

SEQ ID NO: 4 - protein, 688 aa, Macaca fascicularis
SIPIPQKLFGEVTSPLFPKPYPNSFETTTVITVPTGYRVKLVFQHFDLEPSEGCFYDYVKISADKKNLGRFCGQLGSPLGNPPGKKEFLSQGNKMLLTFHTDFSNEENGTIMFYKGFLAYYQAVDLDECASQSESGEKDPQPQCQHLCHNYVGGYFCSCRPGYELQEDRHSCQAECSSELYTEASGYISSLEYPRSYPPDLRCNYSIRVERGLTLHLKFLEPFEIDDHQQVHCPYDQLQIYANGKNIGEFCGKQRPPDFDTSSNAVDLLFFTDESGDSRGWKLRYTTEIIKCPQPKTLDEFTVIQNLQPQYQFRDYFIATCKLGYQLIEGNQVLHSFTAVCQDDGTWHRAMPRCKIKDCGQPRNLPNGAFRYTTTMGVNTYKARIQYYCHEPYYKMQTRAGSKESEQGLYTCTAQGIWKNEQKGEKIPRCLPVCGKPVNPVEQRQQIIGGQKAKMGNFPWQVFTNIHGRGGGALLGDRWILTAAHTLYPKEHEAQSNASLDVFLGHTNVEELMKLANHPIRRVSIHPDYRQDESHNFEGDIALLELENSVTLGPNLLPICLPDNETFYDLGLMGYVSGFGVMEEKIAHDLRFVRLPVANRKDCETWLRGKNRLDVFSQNMFCAGHPSLKQDACQGDAGGVFAVRDPNTDRWIATGIVSWGIGCSKGYGFYTKVLNYVDWIKKEMEEED

SEQ ID NO: 5 - protein, 294 aa, Macaca fascicularis
MWFLTALLLWVPVDGQVDTTKAVITLQPPWVSVFQEETVTLQCEVPRLPGSSSTQWFLNGTATQTSTPSYRITSASVKDSGEYRCQRGPSGRSDPIQLEIHRDWLLLQVSSRVFTEGEPLALRCHAWKDKLVYNVLYYQNGKAFKFFYRNSQLTILKTNISHNGAYHCSGMGKHRYTSAGVSVTVKELFPAPVLNASVTSPLLEGNLVTLSCETKLLLQRPGLQLYFSFYMGSKTLRGRNTSSEYQILTARREDSGFYWCEATTEDGNVLKRSPELELQVLGLQLPTPHHHHHH

SEQ ID NO: 6 - protein, 217 aa, Macaca fascicularis
MSQNVCPGNLWLLQPLTVLLLLASADSQTAPPKAVLKLEPPWINVLREDSVTLTCGGAHSPDSDSTQWFHNGNLIPTHTQPSYRFKANNNDSGEYRCQTGRTSLSDPVHLTVLSEWLALQTPHLEFREGETIMLRCHSWKDKPLIKVTFFQNGIAKKFSHMDPNFSIPRANHSHSGDYHCTGNIGYTPYSSKPVTITVQVPSVGSSSPMGIHHHHHH

SEQ ID NO: 7 - protein, 217 aa, Macaca fascicularis
MSQNVCPGNLWLLQPLTVLLLLASADSQTAPPKAVLKLEPPWINVLREDSVTLTCGGAHSPDSDSTQWFHNGNLIPTHTQPSYRFKANNNDSGEYRCQTGRTSLSDPVHLTVLSEWLALQTTHLEFREGETIMLRCHSWKDKPLIKVAFFQNGKSKNFSHMNPNFSIPQANHSHSGDYHCTGNIGYTPYSSKPVTITVQVPSVGSSSPMGIHHHHHH

SEQ ID NO: 8 - protein, 217 aa, Macaca fascicularis
MSQNVCPGNLWLLQPLTVLLLLASADSQTAPPKAVLKLEPPWINVLREDSVTLTCGGAHSPDSDSTQWFHNGNLIPTHTQPSYRFKANNNDSGEYRCQTGRTSLSDPVHLTVLSEWLALQTTHLEFREGETIMLRCHSWKDKPLIKVAFFQNGISKKFSPMNPNFSIPRANHSHSGDYHCTGNIGYTPYSSKPVTITVQVPSVGSSSPMGIHHHHHH

SEQ ID NO: 9 - protein, 223 aa, Macaca fascicularis
MGILSFLPVLATESDWADCKSSQPWGHMLLWTAVLFLAPVAGTPAAPPKAVLKLEPPWINVLREDSVTLTCGGAHSPDSDSTQWFHNGNLIPTHTQPSYRFKANNNDSGEYRCQTGRTSLSDPVHLTVLSEWLALQTPHLEFREGETIMLRCHSWKDKPLIKVTFFQNGISKKFSHMNPNFSIPQANHSHSGDYHCTGNIGYTPYSSKPVTITVQVPHHHHHH

SEQ ID NO: 10 - protein, 214 aa, Macaca fascicularis
MWQLLLPTALLLLVSAGMRAEDLPKAVVFLEPQWYRVLEKDRVTLKCQGAYSPEDNSTRWFHNESLISSQTSSYFIAAARVNNSGEYRCQTSLSTLSDPVQLEVHIGWLLLQAPRWVFKEEESIHLRCHSWKNTLLHKVTYLQNGKGRKYFHQNSDFYIPKATLKDSGSYFCRGLIGSKNVSSETVNITITQDLAVSSISSFFPPGYQHHHHHH

SEQ ID NO: 11 - protein, 214 aa, Macaca fascicularis
MWQLLLPTALLLLVSAGMRAEDLPKAVVFLEPQWYRVLEKDSVTLKCQGAYSPEDNSTRWFHNESLISSQTSSYFIAAARVNNSGEYRCQTSLSTLSDPVQLEVHIGWLLLQAPRWVFKEEESIHLRCHSWKNTLLHKVTYLQNGKGRKYFHQNSDFYIPKATLKDSGSYFCRGLIGSKNVSSETVNITITQDLAVSSISSFFPPGYQHHHHHH

SEQ ID NO: 12 - protein, 294 aa, Homo sapiens
MWFLTTLLLWVPVDGQVDTTKAVITLQPPWVSVFQEETVTLHCEVLHLPGSSSTQWFLNGTATQTSTPSYRITSASVNDSGEYRCQRGLSGRSDPIQLEIHRGWLLLQVSSRVFTEGEPLALRCHAWKDKLVYNVLYYRNGKAFKFFHWNSNLTILKTNISHNGTYHCSGMGKHRYTSAGISVTVKELFPAPVLNASVTSPLLEGNLVTLSCETKLLLQRPGLQLYFSFYMGSKTLRGRNTSSEYQILTARREDSGLYWCEAATEDGNVLKRSPELELQVLGLQLPTPHHHHHH

SEQ ID NO: 13 - protein, 224 aa, Homo sapiens
MTMETQMSQNVCPRNLWLLQPLTVLLLLASADSQAAAPPKAVLKLEPPWINVLQEDSVTLTCQGARSPESDSIQWFHNGNLIPTHTQPSYRFKANNNDSGEYTCQTGQTSLSDPVHLTVLSEWLVLQTPHLEFQEGETIMLRCHSWKDKPLVKVTFFQNGKSQKFSRLDPTFSIPQANHSHSGDYHCTGNIGYTLFSSKPVTITVQVPSMGSSSPMGIHHHHHH

SEQ ID NO: 14 - protein, 224 aa, Homo sapiens
MTMETQMSQNVCPRNLWLLQPLTVLLLLASADSQAAAPPKAVLKLEPPWINVLQEDSVTLTCQGARSPESDSIQWFHNGNLIPTHTQPSYRFKANNNDSGEYTCQTGQTSLSDPVHLTVLSEWLVLQTPHLEFQEGETIMLRCHSWKDKPLVKVTFFQNGKSQKFSHLDPTFSIPQANHSHSGDYHCTGNIGYTLFSSKPVTITVQVPSMGSSSPMGIHHHHHH

SEQ ID NO: 15 - protein, 223 aa, Homo sapiens
MGILSFLPVLATESDWADCKSPQPWGHMLLWTAVLFLAPVAGTPAAPPKAVLKLEPQWINVLQEDSVTLTCRGTHSPESDSIQWFHNGNLIPTHTQPSYRFKANNNDSGEYTCQTGQTSLSDPVHLTVLSEWLVLQTPHLEFQEGETIVLRCHSWKDKPLVKVTFFQNGKSKKFSRSDPNFSIPQANHSHSGDYHCTGNIGYTLYSSKPVTITVQAPHHHHHH

SEQ ID NO: 16 - protein, 214 aa, Homo sapiens
MWQLLLPTALLLLVSAGMRTEDLPKAVVFLEPQWYRVLEKDSVTLKCQGAYSPEDNSTQWFHNESLISSQASSYFIDAATVDDSGEYRCQTNLSTLSDPVQLEVHIGWLLLQAPRWVFKEEDPIHLRCHSWKNTALHKVTYLQNGKGRKYFHHNSDFYIPKATLKDSGSYFCRGLFGSKNVSSETVNITITQGLAVSTISSFFPPGYQHHHHHH

SEQ ID NO: 17 - protein, 214 aa, Homo sapiens
MWQLLLPTALLLLVSAGMRTEDLPKAVVFLEPQWYRVLEKDSVTLKCQGAYSPEDNSTQWFHNESLISSQASSYFIDAATVDDSGEYRCQTNLSTLSDPVQLEVHIGWLLLQAPRWVFKEEDPIHLRCHSWKNTALHKVTYLQNGKGRKYFHHNSDFYIPKATLKDSGSYFCRGLVGSKNVSSETVNITITQGLAVSTISSFFPPGYQHHHHHH

SEQ ID NO: 18 - protein, 214 aa, Homo sapiens
MWQLLLPTALLLLVSAGMRTEDLPKAVVFLEPQWYRVLEKDSVTLKCQGAYSPEDNSTQWFHNENLISSQASSYFIDAATVDDSGEYRCQTNLSTLSDPVQLEVHVGWLLLQAPRWVFKEEDPIHLRCHSWKNTALHKVTYLQNGKDRKYFHHNSDFHIPKATLKDSGSYFCRGLVGSKNVSSETVNITITQGLAVSTISSFSPPGYQHHHHHH

SEQ ID NO: 19 - protein, 214 aa, Homo sapiens
MWQLLLPTALLLLVSAGMRTEDLPKAVVFLEPQWYSVLEKDSVTLKCQGAYSPEDNSTQWFHNESLISSQASSYFIDAATVNDSGEYRCQTNLSTLSDPVQLEVHIGWLLLQAPRWVFKEEDPIHLRCHSWKNTALHKVTYLQNGKDRKYFHHNSDFHIPKATLKDSGSYFCRGLVGSKNVSSETVNITITQGLAVSTISSFSPPGYQHHHHHH

SEQ ID NO: 20 - protein, 118 aa, Artificial Sequence
  an artificially synthesized sequence
EVMLVESGGGLVKPGGSLRLSCAASGFTFSNYAMSWVRQAPGKGLEWVATISSGGSHTYYLDSVKGRFTISRDNSKDTLYLQMNSLRAEDTALYYCARLFTGYAMDYWGQGTLVTVSS

SEQ ID NO: 21 - protein, 109 aa, Artificial Sequence
  an artificially synthesized sequence
QIVLTQSPATLSLSPGERATLSCTASSSVSSSYLHWYQQKPGKAPKLWIYSTSNLASGVPSRFSGSGSGTDYTLTISSLQPEDFATYYCHQYYRLPPITFGQGTKLEIK

SEQ ID NO: 22 - protein, 328 aa, Artificial Sequence
  an artificially synthesized sequence
ASTKGPSVFPLAPSSKSTSGGTAALGCLVKDYFPEPVTVSWNSGALTSGVHTFPAVLQSSGLYSLSSVVTVPSSSLGTQTYICNVNHKPSNTKVDKKVEPKSCDKTHTCPPCPAPELLGGPSVFLFPPKPKDTLMISRTPEVTCVVVDVSHEDPEVKFNWYVDGVEVHNAKTKPREEQYNSTYRVVSVLTVLHQDWLNGKEYKCEVSNKALPAPIEKTISKAKGQPREPQVYTLPPSREEMTKNQVSLTCLVKGFYPSDIAVEWESNGQPENNYKTTPPVLDSDGSFFLYSKLTVDKSRWQQGNVFSCSVMHEALHNHYTQKSLSLSP

SEQ ID NO: 23 - protein, 107 aa, Artificial Sequence [sequence omitted]

SEQ ID NO: 24 - protein, 120 aa, Artificial Sequence
  an artificially synthesized sequence
QVQLVESGGGVVQPGRSLRLSCAASGFTFSAYAMNWIRQPPGKGLEWIGLIYGSGHEFYASWAEERVTISVDTSKNQFSLKLSSVTAADTAVYYCARGRSKNYNSDFHLWGQGTLVTVSS

SEQ ID NO: 25 - protein, 5 aa, Artificial Sequence
  an artificially synthesized sequence
AYAMN

SEQ ID NO: 26 - protein, 16 aa, Artificial Sequence
  an artificially synthesized sequence
LIYGSGHEFYASWAEE

SEQ ID NO: 27 - protein, 12 aa, Artificial Sequence
  an artificially synthesized sequence
GRSKNYNSDFHL

SEQ ID NO: 28 - protein, 120 aa, Artificial Sequence
  an artificially synthesized sequence
QVQLVESGGGVVQPGRSLRLSCAASGFTFSAYAMNWIRQPPGKGLEWIGLIYGTGHEFYASWAEERVTISVDTSKNQFSLKLSSVTAADTAVYYCARGRSKNYNSDFHIWGQGTLVTVSS

SEQ ID NO: 29 - protein, 5 aa, Artificial Sequence
  an artificially synthesized sequence
AYAMN

SEQ ID NO: 30 - protein, 16 aa, Artificial Sequence
  an artificially synthesized sequence
LIYGTGHEFYASWAEE

SEQ ID NO: 31 - protein, 12 aa, Artificial Sequence
  an artificially synthesized sequence
GRSKNYNSDFHI

SEQ ID NO: 32 - protein, 120 aa, Artificial Sequence
  an artificially synthesized sequence
QVQLVESGGGVVQPGRSLRLSCAASGFTFSAYAMNWIRQPPGKGLEWIGLMYGSGHEFYASWAEERVTISVDTSKNQFSLKLSSVTAADTAVYYCARGRSKNYNSDFHLWGQGTLVTVSS

SEQ ID NO: 33 - protein, 5 aa, Artificial Sequence
  an artificially synthesized sequence
AYAMN

SEQ ID NO: 34 - protein, 16 aa, Artificial Sequence
  an artificially synthesized sequence
LMYGSGHEFYASWAEE

SEQ ID NO: 35 - protein, 12 aa, Artificial Sequence
  an artificially synthesized sequence
GRSKNYNSDFHL

SEQ ID NO: 36 - protein, 120 aa, Artificial Sequence
  an artificially synthesized sequence
QVQLVESGGGVVQPGRSLRLSCAASGFTFSAYTMNWIRQPPGKGLEWIGLIYGSGHEFYASWAEERVTISVDTSKNQFSLKLSSVTAADTAVYYCARGRSKNYNSDFHLWGQGTLVTVSS

SEQ ID NO: 37 - protein, 5 aa, Artificial Sequence
  an artificially synthesized sequence
AYTMN

SEQ ID NO: 38 - protein, 16 aa, Artificial Sequence
  an artificially synthesized sequence
LIYGSGHEFYASWAEE

SEQ ID NO: 39 - protein, 12 aa, Artificial Sequence
  an artificially synthesized sequence
GRSKNYNSDFHL

SEQ ID NO: 40 - protein, 120 aa, Artificial Sequence
  an artificially synthesized sequence
QVQLVESGGGVVQPGRSLRLSCAASGFTFSAYAMNWIRQPPGKGLEWIGLIYGSGHEFYASWAEERVTISVDTSKNQFSLKLSSVTAADTAVYYCARGRSKNYVSGFHLWGQGTLVTVSS

SEQ ID NO: 41 - protein, 120 aa, Artificial Sequence
  an artificially synthesized sequence
QVQLVESGGGVVQPGRSLRLSCAASGFRFSAYAMNWIRQPPGKGLEWIGLIYGKGSTFYASWAKERVTISVDTSKNQFSLKLSSVTAADTAVYYCARGRSVNYNSDFHLWGQGTLVTVSS

SEQ ID NO: 42 - protein, 328 aa, Artificial Sequence
  an artificially synthesized sequence
ASTKGPSVFPLAPSSKSTSGGTAALGCLVKDYFPEPVTVSWNSGALTSGVHTFPAVLQSSGLYSLSSVVTVPSSSLGTQTYICNVNHKPSNTKVDKRVEPKSCDKTHTCPPCPAPELWNGPSVFLFPPKPKDTLMISRTPEVTCVVVDVSDEDPEVKFNWYVDGVEVHNAKTKPREELYNSTYRVVSVLTVLHRDWLNGKEYKCKVSNTALPKPIEKTISKAKGQRREPQVYTLPPSREEMTKNQVSLTCLVKGFYPSDIAVEWESNGQPENNYKTTPPVLDSDGSFFLYSKLTVDKSRWQQGNVFSCSVLHEALHAHTTRKELSLSP

SEQ ID NO: 43 - protein, 328 aa, Artificial Sequence
  an artificially synthesized sequence
ASTKGPSVFPLAPSSKSTSGGTAALGCLVKDYFPEPVTVSWNSGALTSGVHTFPAVLQSSGLYSLSSVVTVPSSSLGTQTYICNVNHKPSNTKVDKRVEPKSCDKTHTCPPCPAPELRRGPSVFLFPPKPKDTLMISRTPEVTCVVVDVSDEDPEVKFNWYVDGVEVHNAKTKPREELYNSTYRVVSVLTVLHRDWLNGKEYKCKVSNTALPKPIEKTISKAKGQRREPQVYTLPPSREEMTKNQVSLTCLVKGFYPSDIAVEWESNGQPENNYKTTPPVLDSDGSFFLYSKLTVDKSRWQQGNVFSCSVLHEALHAHTTRKELSLSP

SEQ ID NO: 44 - protein, 328 aa, Artificial Sequence
  an artificially synthesized sequence
ASTKGPSVFPLAPSSKSTSGGTAALGCLVKDYFPEPVTVSWNSGALTSGVHTFPAVLQSSGLYSLSSVVTVPSSSLGTQTYICNVNHKPSNTKVDKRVEPKSCDKTHTCPPCPAPEYLGGDSVFLFPPKPKDVLMISRTPEVTCVVIDVSHEDPEVKFNWYVDGVEVHNAKTKPREEQYNSTYRVVSVLPVLHRDWLNGKEYKCKVSNKALPKPIEKTISKAKGQRREPQVYTLPPSREEMTKNQVSLTCLVKGFYPSDIAVEWESNGQPENNYKTTPPVLDSDGSFFLYSKLTVDKSRWQQGNVFSCSVLHEALHAHTTRKELSLSP

SEQ ID NO: 45 - protein, 328 aa, Artificial Sequence
  an artificially synthesized sequence
ASTKGPSVFPLAPSSRSTSESTAALGCLVKDYFPEPVTVSWNSGALTSGVHTFPAVLQSSGLYSLSSVVTVPSSSLGTQTYICNVNHKPSNTKVDKRVEPKSCDKTHTCPPCPAPELRRGPSVFLFPPKPKDTLMISRTPEVTCVVVDVSQEDPEVQFNWYVDGVEVHNAKTKPREEQYNSTYRVVSVLTVLHQDWLNGKEYKCKVSNKALPAPIEKTISKAKGQPREPQVYTLPPSQEEMTKNQVSLTCLVKGFYPSDIAVEWESNGQPENNYKTTPPVLDSDGSFFLYSKLTVDKSRWQEGNVFSCSVLHEALHAHTTRKELSLSP

SEQ ID NO: 46 - protein, 113 aa, Artificial Sequence
  an artificially synthesized sequence
DIQMTQSPSSLSASVGDRVTITCQASQSLHDKKNLAWYQQKPGQPPKLLIYGASTLESGVPSRFSGSGSGTDFTLTISSLQPEDFATYYCQGEFSCSSADCNTFGQGTKVEIK

SEQ ID NO: 47 - protein, 113 aa, Artificial Sequence
  an artificially synthesized sequence
DIQMTQSPSSLSASVGDRVTITCQAHEILHDKKNLAWYQQKPGQPPKLLIYSASILESGVPSRFSGSGSGTDFTLTISSLQPEDFATYYCHGEFSHGSGDLNHFGQGTKVEIK

SEQ ID NO: 48 - protein, 13 aa, Artificial Sequence
  an artificially synthesized sequence
QAHEILHDKKNLA

SEQ ID NO: 49 - protein, 7 aa, Artificial Sequence
  an artificially synthesized sequence
SASILES

SEQ ID NO: 50 - protein, 13 aa, Artificial Sequence
  an artificially synthesized sequence
HGEFSHGSGDLNH

SEQ ID NO: 51 - protein, 113 aa, Artificial Sequence
  an artificially synthesized sequence
DIQMTQSPSSLSASVGDRVTITCQAHEILHDKKNLAWYQQKPGQPPKLLIYSASILESGVPSRFSGSGSGTDFTLTISSLQPEDFATYYCHGEFSHGSADLNHFGQGTKVEIK

SEQ ID NO: 52 - protein, 13 aa, Artificial Sequence
  an artificially synthesized sequence
QAHEILHDKKNLA

SEQ ID NO: 53 - protein, 7 aa, Artificial Sequence
  an artificially synthesized sequence
SASILES

SEQ ID NO: 54 - protein, 13 aa, Artificial Sequence
  an artificially synthesized sequence
HGEFSHGSADLNH

SEQ ID NO: 55 - protein, 113 aa, Artificial Sequence
  an artificially synthesized sequence
DIQMTQSPSSLSASVGDRVTITCQAHEILHDKKNLAWYQQKPGQPPKLLIYGASQRESGVPSRFSGSGSGTDFTLTISSLQPEDFATYYCHGEFPHSSADLNHFGQGTKVEIK

SEQ ID NO: 56 - protein, 13 aa, Artificial Sequence
  an artificially synthesized sequence
QAHEILHDKKNLA

SEQ ID NO: 57 - protein, 7 aa, Artificial Sequence
  an artificially synthesized sequence
GASQRES

SEQ ID NO: 58 - protein, 13 aa, Artificial Sequence
  an artificially synthesized sequence
HGEFPHSSADLNH

SEQ ID NO: 59 - protein, 113 aa, Artificial Sequence
  an artificially synthesized sequence
DIQMTQSPSSLSASVGDRVTITCQANEILHDKKNLAWYQQKPGQPPKLLIYGASTLESGVPSRFSGSGSGTDFTLTISSLQPEDFATYYCHGEFSYHSADLNTFGQGTKVEIK

SEQ ID NO: 60 - protein, 13 aa, Artificial Sequence
  an artificially synthesized sequence
QANEILHDKKNLA

SEQ ID NO: 61 - protein, 7 aa, Artificial Sequence
  an artificially synthesized sequence
GASTLES

SEQ ID NO: 62 - protein, 13 aa, Artificial Sequence
  an artificially synthesized sequence
HGEFSYHSADLNT

SEQ ID NO: 63 - protein, 113 aa, Artificial Sequence
  an artificially synthesized sequence
DIQMTQSPSSLSASVGDRVTITCQANQILHDKKNLAWYQQKPGQPPKLLIYGASTLESGVPSRFSGSGSGTDFTLTISSLQPEDFATYYCHGEFSYSSADLNTFGQGTKVEIK

SEQ ID NO: 64 - protein, 113 aa, Artificial Sequence
  an artificially synthesized sequence
DIQMTQSPSSLSASVGDRVTITCQASQILHDKKNLAWYQQKPGQPPKLLIYQASQLESGVPSRFSGSGSGTDFTLTISSLQPEDFATYYCHGEFSYESADLNQFGQGTKVEIK

SEQ ID NO: 65 - protein, 328 aa, Artificial Sequence
  an artificially synthesized sequence
ASTKGPSVFPLAPSSKSTSGGTAALGCLVKDYFPEPVTVSWNSGALTSGVHTFPAVLQSSGLYSLSSVVTVPSSSLGTQTYICNVNHKPSNTKVDKKVEPKSCDKTHTCPPCPAPELLGGPSVFLFPPKPKDTLMISRTPEVTCVVVDVSHEDPEVKFNWYVDGVEVHNAKTKPREEQYNSTYRVVSVLTVLHQDWLNGKEYKCKVSNKALPAPIEKTISKAKGQPREPQVYTLPPSREEMTKNQVSLTCLVKGFYPSDIAVEWESNGQPENNYKTTPPVLDSDGSFFLYSKLTVDKSRWQQGNVFSCSVMHEALHNHYTQKSLSLSP

SEQ ID NO: 66 - protein, 448 aa, Artificial Sequence
  an artificially synthesized sequence
QVQLVESGGGVVQPGRSLRLSCAASGFTFSAYAMNWIRQPPGKGLEWIGLIYGSGHEFYASWAEERVTISVDTSKNQFSLKLSSVTAADTAVYYCARGRSKNYNSDFHLWGQGTLVTVSSASTKGPSVFPLAPSSRSTSESTAALGCLVKDYFPEPVTVSWNSGALTSGVHTFPAVLQSSGLYSLSSVVTVPSSSLGTQTYICNVNHKPSNTKVDKRVEPKSCDKTHTCPPCPAPELRRGPSVFLFPPKPKDTLMISRTPEVTCVVVDVSQEDPEVQFNWYVDGVEVHNAKTKPREEQYNSTYRVVSVLTVLHQDWLNGKEYKCKVSNKALPAPIEKTISKAKGQPREPQVYTLPPSQEEMTKNQVSLTCLVKGFYPSDIAVEWESNGQPENNYKTTPPVLDSDGSFFLYSKLTVDKSRWQEGNVFSCSVLHEALHAHTTRKELSLSP

SEQ ID NO: 67 - protein, 220 aa, Artificial Sequence
  an artificially synthesized sequence
DIQMTQSPSSLSASVGDRVTITCQANEILHDKKNLAWYQQKPGQPPKLLIYGASTLESGVPSRFSGSGSGTDFTLTISSLQPEDFATYYCHGEFSYHSADLNTFGQGTKVEIKRTVAAPSVFIFPPSDEQLKSGTASVVCLLNNFYPREAKVQWKVDNALQSGNSQESVTEQDSKDSTYSLSSTLTLSKADYEKHKVYACEVTHQGLSSPVTKSFNRGEC

SEQ ID NO: 68 - protein, 448 aa, Artificial Sequence
  an artificially synthesized sequence
QVQLVESGGGVVQPGRSLRLSCAASGFTFSAYTMNWIRQPPGKGLEWIGLIYGSGHEFYASWAEERVTISVDTSKNQFSLKLSSVTAADTAVYYCARGRSKNYNSDFHLWGQGTLVTVSSASTKGPSVFPLAPSSRSTSESTAALGCLVKDYFPEPVTVSWNSGALTSGVHTFPAVLQSSGLYSLSSVVTVPSSSLGTQTYICNVNHKPSNTKVDKRVEPKSCDKTHTCPPCPAPELRRGPSVFLFPPKPKDTLMISRTPEVTCVVVDVSQEDPEVQFNWYVDGVEVHNAKTKPREEQYNSTYRVVSVLTVLHQDWLNGKEYKCKVSNKALPAPIEKTISKAKGQPREPQVYTLPPSQEEMTKNQVSLTCLVKGFYPSDIAVEWESNGQPENNYKTTPPVLDSDGSFFLYSKLTVDKSRWQEGNVFSCSVLHEALHAHTTRKELSLSP

SEQ ID NO: 69 - protein, 220 aa, Artificial Sequence
  an artificially synthesized sequence
DIQMTQSPSSLSASVGDRVTITCQAHEILHDKKNLAWYQQKPGQPPKLLIYGASQRESGVPSRFSGSGSGTDFTLTISSLQPEDFATYYCHGEFPHSSADLNHFGQGTKVEIKRTVAAPSVFIFPPSDEQLKSGTASVVCLLNNFYPREAKVQWKVDNALQSGNSQESVTEQDSKDSTYSLSSTLTLSKADYEKHKVYACEVTHQGLSSPVTKSFNRGEC

SEQ ID NO: 70 - protein, 448 aa, Artificial Sequence; identical to SEQ ID NO: 66
  an artificially synthesized sequence

SEQ ID NO: 71 - protein, 220 aa, Artificial Sequence; identical to SEQ ID NO: 69
  an artificially synthesized sequence

SEQ ID NO: 72 - protein, 448 aa, Artificial Sequence; identical to SEQ ID NO: 66
  an artificially synthesized sequence

SEQ ID NO: 73 - protein, 220 aa, Artificial Sequence
  an artificially synthesized sequence
DIQMTQSPSSLSASVGDRVTITCQAHEILHDKKNLAWYQQKPGQPPKLLIYSASILESGVPSRFSGSGSGTDFTLTISSLQPEDFATYYCHGEFSHGSGDLNHFGQGTKVEIKRTVAAPSVFIFPPSDEQLKSGTASVVCLLNNFYPREAKVQWKVDNALQSGNSQESVTEQDSKDSTYSLSSTLTLSKADYEKHKVYACEVTHQGLSSPVTKSFNRGEC

SEQ ID NO: 74 - protein, 448 aa, Artificial Sequence
  an artificially synthesized sequence
QVQLVESGGGVVQPGRSLRLSCAASGFTFSAYAMNWIRQPPGKGLEWIGLIYGTGHEFYASWAEERVTISVDTSKNQFSLKLSSVTAADTAVYYCARGRSKNYNSDFHIWGQGTLVTVSSASTKGPSVFPLAPSSRSTSESTAALGCLVKDYFPEPVTVSWNSGALTSGVHTFPAVLQSSGLYSLSSVVTVPSSSLGTQTYICNVNHKPSNTKVDKRVEPKSCDKTHTCPPCPAPELRRGPSVFLFPPKPKDTLMISRTPEVTCVVVDVSQEDPEVQFNWYVDGVEVHNAKTKPREEQYNSTYRVVSVLTVLHQDWLNGKEYKCKVSNKALPAPIEKTISKAKGQPREPQVYTLPPSQEEMTKNQVSLTCLVKGFYPSDIAVEWESNGQPENNYKTTPPVLDSDGSFFLYSKLTVDKSRWQEGNVFSCSVLHEALHAHTTRKELSLSP

SEQ ID NO: 75 - protein, 220 aa, Artificial Sequence
  an artificially synthesized sequence
DIQMTQSPSSLSASVGDRVTITCQAHEILHDKKNLAWYQQKPGQPPKLLIYSASILESGVPSRFSGSGSGTDFTLTISSLQPEDFATYYCHGEFSHGSADLNHFGQGTKVEIKRTVAAPSVFIFPPSDEQLKSGTASVVCLLNNFYPREAKVQWKVDNALQSGNSQESVTEQDSKDSTYSLSSTLTLSKADYEKHKVYACEVTHQGLSSPVTKSFNRGEC

SEQ ID NO: 76 - protein, 448 aa, Artificial Sequence
  an artificially synthesized sequence
QVQLVESGGGVVQPGRSLRLSCAASGFTFSAYAMNWIRQPPGKGLEWIGLMYGSGHEFYASWAEERVTISVDTSKNQFSLKLSSVTAADTAVYYCARGRSKNYNSDFHLWGQGTLVTVSSASTKGPSVFPLAPSSRSTSESTAALGCLVKDYFPEPVTVSWNSGALTSGVHTFPAVLQSSGLYSLSSVVTVPSSSLGTQTYICNVNHKPSNTKVDKRVEPKSCDKTHTCPPCPAPELRRGPSVFLFPPKPKDTLMISRTPEVTCVVVDVSQEDPEVQFNWYVDGVEVHNAKTKPREEQYNSTYRVVSVLTVLHQDWLNGKEYKCKVSNKALPAPIEKTISKAKGQPREPQVYTLPPSQEEMTKNQVSLTCLVKGFYPSDIAVEWESNGQPENNYKTTPPVLDSDGSFFLYSKLTVDKSRWQEGNVFSCSVLHEALHAHTTRKELSLSP

SEQ ID NO: 77 - protein, 220 aa, Artificial Sequence; identical to SEQ ID NO: 69
  an artificially synthesized sequence

SEQ ID NO: 78 - protein, 448 aa, Artificial Sequence
  an artificially synthesized sequence
QVQLVESGGGVVQPGRSLRLSCAASGFTFSAYAMNWIRQPPGKGLEWIGLIYGSGHEFYASWAEERVTISVDTSKNQFSLKLSSVTAADTAVYYCARGRSKNYNSDFHLWGQGTLVTVSSASTKGPSVFPLAPSSKSTSGGTAALGCLVKDYFPEPVTVSWNSGALTSGVHTFPAVLQSSGLYSLSSVVTVPSSSLGTQTYICNVNHKPSNTKVDKRVEPKSCDKTHTCPPCPAPEYLGGDSVFLFPPKPKDVLMISRTPEVTCVVIDVSHEDPEVKFNWYVDGVEVHNAKTKPREEQYNSTYRVVSVLPVLHRDWLNGKEYKCKVSNKALPKPIEKTISKAKGQRREPQVYTLPPSREEMTKNQVSLTCLVKGFYPSDIAVEWESNGQPENNYKTTPPVLDSDGSFFLYSKLTVDKSRWQQGNVFSCSVLHEALHAHTTRKELSLSP

SEQ ID NO: 79 - protein, 220 aa, Artificial Sequence; identical to SEQ ID NO: 67
  an artificially synthesized sequence

SEQ ID NO: 80 - protein, 448 aa, Artificial Sequence
  an artificially synthesized sequence
QVQLVESGGGVVQPGRSLRLSCAASGFTFSAYTMNWIRQPPGKGLEWIGLIYGSGHEFYASWAEERVTISVDTSKNQFSLKLSSVTAADTAVYYCARGRSKNYNSDFHLWGQGTLVTVSSASTKGPSVFPLAPSSKSTSGGTAALGCLVKDYFPEPVTVSWNSGALTSGVHTFPAVLQSSGLYSLSSVVTVPSSSLGTQTYICNVNHKPSNTKVDKRVEPKSCDKTHTCPPCPAPEYLGGDSVFLFPPKPKDVLMISRTPEVTCVVIDVSHEDPEVKFNWYVDGVEVHNAKTKPREEQYNSTYRVVSVLPVLHRDWLNGKEYKCKVSNKALPKPIEKTISKAKGQRREPQVYTLPPSREEMTKNQVSLTCLVKGFYPSDIAVEWESNGQPENNYKTTPPVLDSDGSFFLYSKLTVDKSRWQQGNVFSCSVLHEALHAHTTRKELSLSP

SEQ ID NO: 81 - protein, 220 aa, Artificial Sequence; identical to SEQ ID NO: 69
  an artificially synthesized sequence

SEQ ID NO: 82 - protein, 448 aa, Artificial Sequence; identical to SEQ ID NO: 78
  an artificially synthesized sequence

SEQ ID NO: 83 - protein, 220 aa, Artificial Sequence; identical to SEQ ID NO: 69
  an artificially synthesized sequence

SEQ ID NO: 84 - protein, 448 aa, Artificial Sequence; identical to SEQ ID NO: 78
  an artificially synthesized sequence

SEQ ID NO: 85 - protein, 220 aa, Artificial Sequence; identical to SEQ ID NO: 73
  an artificially synthesized sequence

SEQ ID NO: 86 - protein, 448 aa, Artificial Sequence
  an artificially synthesized sequence
QVQLVESGGGVVQPGRSLRLSCAASGFTFSAYAMNWIRQPPGKGLEWIGLIYGTGHEFYASWAEERVTISVDTSKNQFSLKLSSVTAADTAVYYCARGRSKNYNSDFHIWGQGTLVTVSSASTKGPSVFPLAPSSKSTSGGTAALGCLVKDYFPEPVTVSWNSGALTSGVHTFPAVLQSSGLYSLSSVVTVPSSSLGTQTYICNVNHKPSNTKVDKRVEPKSCDKTHTCPPCPAPEYLGGDSVFLFPPKPKDVLMISRTPEVTCVVIDVSHEDPEVKFNWYVDGVEVHNAKTKPREEQYNSTYRVVSVLPVLHRDWLNGKEYKCKVSNKALPKPIEKTISKAKGQRREPQVYTLPPSREEMTKNQVSLTCLVKGFYPSDIAVEWESNGQPENNYKTTPPVLDSDGSFFLYSKLTVDKSRWQQGNVFSCSVLHEALHAHTTRKELSLSP

SEQ ID NO: 87 - protein, 220 aa, Artificial Sequence; identical to SEQ ID NO: 75
  an artificially synthesized sequence

SEQ ID NO: 88 - protein, 448 aa, Artificial Sequence
  an artificially synthesized sequence
QVQLVESGGGVVQPGRSLRLSCAASGFTFSAYAMNWIRQPPGKGLEWIGLMYGSGHEFYASWAEERVTISVDTSKNQFSLKLSSVTAADTAVYYCARGRSKNYNSDFHLWGQGTLVTVSSASTKGPSVFPLAPSSKSTSGGTAALGCLVKDYFPEPVTVSWNSGALTSGVHTFPAVLQSSGLYSLSSVVTVPSSSLGTQTYICNVNHKPSNTKVDKRVEPKSCDKTHTCPPCPAPEYLGGDSVFLFPPKPKDVLMISRTPEVTCVVIDVSHEDPEVKFNWYVDGVEVHNAKTKPREEQYNSTYRVVSVLPVLHRDWLNGKEYKCKVSNKALPKPIEKTISKAKGQRREPQVYTLPPSREEMTKNQVSLTCLVKGFYPSDIAVEWESNGQPENNYKTTPPVLDSDGSFFLYSKLTVDKSRWQQGNVFSCSVLHEALHAHTTRKELSLSP

SEQ ID NO: 89 - protein, 220 aa, Artificial Sequence; identical to SEQ ID NO: 69
  an artificially synthesized sequence